European Patent Specification EP 3 665 309 B1, published February 22, 2023. Title: COMPOSITIONS AND METHODS FOR DETECTING STAPHYLOCOCCUS AUREUS. Applicant: Gen-Probe Incorporated. The sequence listing filed with the application follows.

SEQUENCE LISTING (126 sequences)

SEQ ID NO: 1 - DNA, 709 bp, Staphylococcus aureus
tacattagaaatacaaggaaagatgctatcttccgaaggattggcccaagaattgaaccaacgcatgacccaagggcaaagcgactttgttttcgtcattggcggatcaaacggcctgcacaaggacgtcttacaacgcagtaactacgcactatcattcagcaaaatgacattcccacatcaaatgatgcgggttgtgttaattgaacaagtgtacagagcatttaagattatgcgaggagaagcttatcataagtaatgaggttcatgatttttgacatagttagcctccgcagtctttcatttcaagtaaataatagcgaaatattctttatactgaatacttatagtgaagcaaagttctagctttgagaaaattctttctgcaactaaatatagtaaattacggtaaaatataaataagtacatattgaagaaaatgagacataatatattttataataggagggaatttcaaatgatagacaactttatgcaggtccttaaattaattaaagagaaacgtaccaataatgtagttaaaaaatctgattgggataaaggtgatctatataaaactttagtccatgataagttacccaagcagttaaaagtgcatataaaagaagataaatattcagttgtagggaaggttgctactgggaactatagtaaagttccttggatttcaatatatgatgagaatata

SEQ ID NO: 2 - DNA, 980 bp, Staphylococcus aureus
taaatgtcaggaaaatatcaaaaactgcaaaaaatattggtataataagagggaacagtgtgaacaagttaataacttgtggataactggaaagttgataacaatttggaggaccaaacgacatgaaaatcaccattttagctgtagggaaactaaaagagaaatattggaagcaagccatagcagaatatgaaaaacgtttaggcccatacaccaagatagacatcatagaagttccagacgaaaaagcaccagaaaatatgagcgacaaagaaattgagcaagtaaaagaaaaagaaggccaacgaatactagccaaaattaaaccacaatccacagtcattacattagaaatacaaggaaagatgctatcttccgaaggattggcccaagaattgaaccaacgcatgacccaagggcaaagcgactttgtattcgtcattggcggatcaaacggcctgcacaaggacgtcttacaacgcagtaactacgcactatcattcagcaaaatgacattcccacatcaaatgatgcgggttgtgttaattgagcaagtgtatagagcatttaagattatgcgtggagaagcatatcataaatgatgcggttttttcagccgcttcataaagggattttgaatgtatcagaacatatgaggtttatgtgaattgctgttatgtttttaagaagcttatcataagtaatgaggttcatgatttttgacatagttagcctccgcagtctttcatttcaagtaaataatagcgaaatattctttatactgaatacttatagtgaagcaaagttctagctttgagaaaattctttctgcaactaaatatagtaaattacggtaaaatataaataagtacatattgaagaaaatgagacataatatattttataataggagggaatttcaaatgatagacaactttatgcaggtccttaaattaattaaagagaaacgtaccaataat

SEQ ID NO: 3 - DNA, 782 bp, Staphylococcus aureus
caatgcccacagagttatccacaaatacacaggttatacactaaaaattgggcatgaatgtcagaaaaatatcaaaaactgcaaagaatattggtataataagagggaacagtgtgaacaagttaataacttgtggataactggaaagttgataacaatttggaggaccaaacgacatgaaaatcaccattttagctgtagggaaactaaaagagaaatattggaagcaagccatagcagaatatgaaaaacgtttaggcccatacaccaagatagacatcatagaagttccagacgaaaaagcaccagaaaatatgagcgacaaagaaattgagcaagtaaaagaaaaagaaggccaacgaatactagccaaaatcaaaccacaatcaacagtcattacattagaaatacaaggaaagatgctatcttccgaaggattggcccaagaattgaaccaacgcatgacccaagggcaaagcgactttgtattcgtcattggcggatcaaacggcctgcacaaggacgtcttacaacgcagtaactacgcactatcattcagcaaaatgacattcccacatcaaatgatgcgggttgtgttaattgaacaagtgtacagagcatttaagattatgcgtggagaagcgtatcataaataaaactaaaaattaggttgtgtataatttaaaaatttaatgagatgtggaggaattacatatatgaaatattggattataccttgcaatatcatacgatgtttatagagtgtttaataaaccattttt

SEQ ID NO: 4 - DNA, 2153 bp, Staphylococcus aureus
ctgtagggaaactaaaagagaaatactggaagcaagccatagcagaatatgaaaaacgtttaggcccatacaccaagatagacatcatagaagttccagacgaaaaagcaccagaaaatatgagcgacaaagaaatcgagcaagtaaaagaaaaagaaggccaacgaatactagccaaaatcaaaccacaatccacagtcattacattagaaatacaaggaaagatgctatcttccgaaggattggcccaagaattgaaccaacgcatgacccaagggcaaagcgactttgtattcgtcattggcggatcaaacggcctgcacaaggacgtcttacaacgcagtaactacgcactatcattcagcaaaatgacattcccacatcaaatgatgcgggttgtgttaattgaacaagtgtacagagcatttaagattatgcgtggagaagcgtaccacaaatgatgcggttttttatccagttttttgtttaatgaacaaggtaaattacgagataatatttgaagaaaacaataaagtagagatggatttccatatcctctttagtagcggtttttatctgtaaggtttattaataattaaataaataggcgggatagttatatatagcttattaatgaaagaatatgattattaatttagtattatattttaatattaaaaagaagatatgaaataattattcataccttccaccttacaataattagttttcaatcgaatattaagattattagtagtcttaaaagttaagacttccttatattaatgacctaatttattatttgcctcatgaattatctttttatttctttgatatgtcccaaaccacatcgtgatatacactacaataaatattatgatgaaactaataatattctcaaagttcagatggaaccaacctgctagaatagcgagtgggaagaataggattatcatcaatataaagtgaactacagtctgttttgttatactccaatcggtatctgtaaatatcaaattaccataagtaaacaaaattccaatcaatgcccatagtgctacacatattagcataataaccgcttcattaaagttttcataataaattttacccataaaagaatctggatatagtggtacatatttatcccttgaaaaaaataagtgaagtaatgacagaaatcataagaccagtgaacgcacctttttgaacagcgtggaataattttttcatagtgagatggaccattccatttgtttctaacttcaagtgatcaatgtaatttagattgataatttctgattttgaaatacgcacgaatattgaaccgacaagctcttcaatttggtaaagtcgctgataaagttttaaagctttattattcattgttatcgcatacctgtttatcttctactatgaactgtgcaatttgttctagatcaattgggtaaacatgatggttctgttgcaaagtaaaaaaatatagctaaccactaatttatcatgtcagtgttcgcttaacttgctagcatgatgctaatttcgtggcatggcgaaaatccgtagatctgatgagacctgcggttctttttatatagagcgtaaatacattcaataccttttaaagtattctttgctgtattgatactttgataccttgtctttcttactttaatatgacggtgatcttgctcaatgaggttattcaaatatttcgatgtacaatgacagtcaggtttaagtttaaaagctttaattactttagccattgctaccttcgttgaaggtgcctgatctgtaattaccttttgaggtttaccaaattgtttaatgagacgtttaataaacgcatatgctgaatgattatctcgttgcttacgcaaccaaatatctaatgtatgtccctctgcatcaatggcacgatataaatagctccattttccttttattttgatgtacgtctcatcaatacgccatttgtaataagcttttttatgctttttcttccaaatttgatataaaattggggcatattcttgaacccaacggtagaccgttgaatgatgaacgtttacaccacgtccccttaatatttcagatatatcacgataactcaatgcatatcttagatagtagccaacggctacagtgat

SEQ ID NO: 5 - DNA, 1696 bp, Staphylococcus aureus
aaagagaaatattggaagcaagccatagcagaatatgaaaaacgtttaggcccatacaccaagatagacatcatagaagttccagacgaaaaagcaccagaaaatatgagtgacaaagaaattgagcaagtaaaagaaaaagaaggccaacgaatactagccaaaatcaaaccacaatccacagtcattacattagaaatacaaggaaagatgctatcttccgaaggattggcccaagaattgaaccaacgcatgacccaagggcaaagcgactttgttttcgtcattggcggatcaaacggcctgcacaaggacgtcttacaacgcagtaactacgcactatcattcagcaaaatgacattcccacatcaaatgatgcgggttgtgttaattgaacaagtgtacagagcatttaagattatgcgaggagaagcatatcataaatgatgcggttatttcagccgtaattttataatataaagcagagtttattaaattttaatgattactttttattaagaattaattctagttgatatattataatgtgaaacacaaaataataatttgtaattgttagtttataggcatctgtatttggaattttttgtagactatttaaaaaatagtgtatataagtattgagttcatgtattaactgtcttttttcatcgttcatcaagtataaggatgtagagatttgttggataatttcttcggatgtttttaaaattatcattaaattagatggtatctgatcttgagttttgtttttagtgtatgtatattttaaaaaatttttgattgttgttatttgactctcttttaatttgacaccctcatcaataaatgtgttaaatatatcttcatttgtacttaaatcatcaaaatttgccaacaaatatttgaacgtctctaaatcattatgtttgagttccgttttgctattccataattccaaaccatttggtagaaagcccaagctgtgattttgatctccccatatagctgaatttaaatcagtgagttgattaattttttcaacacagaaatgtaattttggaatgaggaatcgaagttgttcttctacttgctgtacttttcttttgttttcaataaaatttctacaccatactgttatcaaaccgccaattattgtgcacaatcctccaatgattgtagataaaattgacaatatattacacacctttcttagaggtttattaacatctatttttgaatttaaaattattactttggtagcgttataacctatttaacagattagagaaaaattgaatgatcgattgaagaatttccaaaataccgtcccatatgcgttgaaggagatttctattttcttctgtattcaaatctttggctttatcctttgctttattcaataaatcatctgagtttttttcaatattttttaatacatctttggcattttgtttaaatactttaggatcggaagttagggcattagagtttgccacattaatcatattattattaatcatttgaatttgattatctgataatatctctgataacctacgctcatcgaggactttattaacagtgtcttcaacttgttgttgtgtgatttgtttatcttgattttgtttaatatctgcaagttgttctttaatatctgctatagaagcatttaaagcttcatctgaatacccat

SEQ ID NO: 6 - DNA, 991 bp, Staphylococcus aureus
accattttagctgtagggaaactaaaagagaaatactggaagcaagccatagcagaatatgaaaaacgtttaggcccatacaccaagatagacatcatagaagttccagacgaaaaagcaccagaaaatatgaactacaaagaaattgagcaagtaaaagaaaaagaaggccaacgaatactagccaaaatcaaaccacaatcaacagtcattacattagaaatacaaggaaagatgctatcttccgaaggattggcccaagaattgaaccaacgcatgacccaagggcaaagcgactttgtattcgtcattggcggatcaaacggcctgcacaaggacgtcttacaacgcagtaactacgcactatcattcagcaaaatgacattcccacatcaaatgatgcgggttgtgttaattgaacaagtgtacagagcatttaagattatgcgaggagaagcgtatcataagtgatggtaaaaaatatgagtaagtagatgaagagtgaaaatcagattaattaataataatgtatcaaatttaaataaaggggtttttaagtatgaatttaagaggtcatgaaaatagacttaaatttcatgcgaaatatgatgtgacacctatatcacatttaaaattattagaaggtcaaaagaaagacggtgaaggcggcatactgacagatagctattactgtttttcatacagcttaaaaggtaattctaaaaaagttttaggtacgtttaattgtggttatcatattgctgaagatttactaaaattatcaaatcaagataaattacctttatttaacccgtttaaagtaattaatgaaggtaatcaattgcagggcgtaacgaataaaggtaatttaaatattaataggcaaagaaaacagtataatgaagtggctttacagctttcaaatgctattaatttaatcataatttgttatgaggataatattaaagaaccactttcaacgataaaatac

SEQ ID NO: 7 - DNA, 1108 bp, Staphylococcus aureus
accattttagctgtagggaaactaaaagagaaatattggaagcaagccatagcagaatatgaaaaacgtttaggcccatacaccaagatagacatcatagaagttccagacgaaaaagcaccagaaaatatgagcgacaaagaaattgagcaagtaaaagaaaaagaaggccaacgaatactagccaaaatcaaaccacaatccacagtcattacattagaaatacaaggaaagatgctatcttccgaaggattggcccaagaattgaaccaacgcatgacccaagggcaaagcgactttgtattcgtcattggcggatcaaacggcctgcacaaggacgtcttacaacgcagtaactatgcactatcatttagcaaaatgacattcccacatcaaatgatgcgggttgtgttaattgaacaagtgtatagagcatttaagattatgcgtggagaagcgtaccacaaataaaactaaaaaatatgagaaaattattaaattagctcaaatctttgaagaataaaaagtgaatattaagtttgataatttaggtacaagtaaagattaagaatttccattatttaatacatggtgtgtaaatcgacttctttttgtattagatgtttgcagtaagcgatgtaaagaagatgctaataaatatgtgaggaatgattacgatactagataagcggctaatgaaattttttaaagtacatatatagacatatttttcatttagtaaaattttgaatttcactttgctaagactagtgtctagaaatttataatgatttattaacacctatttgaaacttaagtataataaatgattcggattttatttttaataaagacaaacttgaacgtagcaaagtagtttttatgataaataataagttttaataatgtgacgcttttatataagcacattattatgaacaatgtgaattgagcatctacaattacattaataaatatataaatgatgatttaaattcacatatatttataatacacatactatatgaaagttttgattatccgaataaatgctaaaattaataaaataattaaaggaatcatacttattatacgtatacgtttagct

SEQ ID NO: 8 - DNA, 1256 bp, Staphylococcus aureus
gctgtagggaaactaaaagagaaatattggaagcaagccatagcagaatatgaaaaacgtttaggcccatacaccaagatagacatcatagaagttccagacgaaaaagcaccagaaaatatgagcgacaaagaaattgagcaagtaaaagaaaaagaaggccaacgaatactagccaaaattaaaccacaatccacagtcattacattagaaatacaaggaaagatgctatcttccgaaggattggcccaagaattgaaccaacgcatgacccaagggcaaagcgactttgtattcgtcattggcggatcaaacggcctgcacaaggacgtcttacaacgcagtaactacgcactatcattcagcaaaatgacattcccacatcaaatgatgcgggttgtgttaattgagcaagtgtatagagcatttaagattatgcgtggagaagcatatcataaatgatgcggttttttcagccgcttcataaagggattttgaatgtatcagaacatatgaggtttatgtgaattgctgttatgtttttaagaagcatatcataagtgatgcggtttttattaattagttgctaaaaaatgaagtatgcaatattaattattattaaattttgatatatttaaagaaagattaagtttagggtgaatgaatggcttatcaaagtgaatatgcattagaaaatgaagtacttcaacaacttgaggaattgaactatgaaagagtaaatatacataatattaaattagaaattaatgaatatctcaaagaactaggagtgttgaaaaatgaataagcagacaaatactccagaactaagatttccagagtttgatgaggaatggaaaaaaaggaaattaggtgaagtagtaaattataaaaatggtggttcatttgaaagtttagtgaaaaaccatggtgtatataaactcataactcttaaatctgttaatacagaaggaaagttgtgtaattctggaaaatatatcgatgataaatgtgttgaaacattgtgtaatgatactttagtaatgatactgagcgagcaagcaccaggactagttggaatgactgcaattatacctaataataatgagtatgtactaaatcaacgagtagcagcactagtgcctaaacaatttatagatagtcaatttctatctaagttaattaatagaaaccagaaatatttcagtgtgagatctgctggaacaaaagtgaaaaatatttctaaaggacatgta

SEQ ID NO: 9 - DNA, 1125 bp, Staphylococcus aureus
accattttagctgtagggaaactaaaagagaaatattggaagcaagccatagcagaatatgaaaaacgtttaggcccatacaccaagatagacatcatagaagttccagacgaaaaagcaccagaaaatatgagcgacaaagaaattgagcaagtaaaagaaaaagaaggccaacgaatactagccaaaatcaaaccacaatccacagtcattacattagaaatacaaggaaagatgctatcttccgaaggattggcccaagaattgaaccaacgcatgacccaagggcaaagcgactttgtattcgtcattggcggatcaaacggcctgcacaaggacgtcttacaacgcagtaactatgcactatcatttagcaaaatgacattcccacatcaaatgatgcgggttgtgttaattgaacaagtgtatagagcatttaagattatgcgtggagaggcgtatcataaataaaactaaaaaacggattgtgtataatatattttaaatataaaaaggattgattttatgttaaataaattagaaaatgttagttataaatcattcgataattacactagtgaagatgatttgactaaagtaaatatattttttggaagaaatgggagtggaaaaagctcattaagtgaatggttaagaagactagataatgaaaaaagtgttatctttaatactggttacttaaaaaataatattgaagaagttgaagaaatagatggtgtgaatttggttattggagaagaatctataaatcatagtgaccaaattaagcatttaaatagcgctataaatagtttagaaaattttattactcggaaaaatagtgaacttaagcattcaaaagaaagaatttacaataaaatgaatatcagactaaatgaagctagagaaagatttgaaataggtagtaatgtggttaagcagaagaggaatgctgacaaagatccagttaatgctttttatagttggaagaaaaatgctaacgatataattcaagagatgactattgaatctttagatgaattagaagaaagaataacaagaaaagaagtcttattaaataatataaaaacaccaattttagcttttgattataatgattttagt

SEQ ID NO: 10 - DNA, 1380 bp, Staphylococcus aureus
accattttagctgtagggaaactaaaagagaaatattggaagcaagccatagcagaatatgaaaaacgtttaggcccatacaccaagatagacatcatagaagttccagacgaaaaagcaccagaaaatatgagcgacaaagaaattgagcaagtaaaagaaaaagaaggccaacgaatactagccaaaattaaaccacaatccacagtcattacattagaaatacaaggaaagatgctatcttccgaaggattggcccaagaattgaaccaacgcatgacccaagggcaaagcgactttgtattcgtcattggcggatcaaacggcctgcacaaggacgtcttacaacgcagtaactacgcactatcattcagcaaaatgacattcccacatcaaatgatgcgggttgtgttaattgagcaagtgtatagagcatttaagattatgcgtggagaagcatatcataagtgatgcggtttttattaattagttgctaaaaaatgaagtatgcaatattaattattattaaattttgatatatttaaagaaagattaagtttagggtgaatgaatggcttatcaaagtgaatatgcattagaaaatgaagtacttcaacaacttgaggaattgaactatgaaagagtaaatatacataatattaaattagaaattaatgaatatctcaaagaactaggagtgttgaaaaatgaataagcagacaaatactccagaactaagatttccagagtttgatgaggaatggaaaaaaaggaaattaggtgaagtagtaaattataaaaatggtggttcatttgaaagtttagtgaaaaaccatggtgtatataaactcataactcttaaatctgttaatacagaaggaaagttgtgtaattctggaaaatatatcgatgataaatgtgttgaaacattgtgtaatgatactttagtaatgatactgagcgagcaagcaccaggactagttggaatgactgcaattatacctaataataatgagtatgtactaaatcaacgagtagcagcactagtgcctaaacaatttatagatagtcaatttctatctaagttaattaatagaaaccagaaatatttcagtgtgagatctgctggaacaaaagtgaaaaatatttctaaaggacatgtagaaaactttaattttttatctcctaattacactgaacaacaaaaaataggtaatttcttcagcaaactcgaccgccagattgagttagaagaagagaaacttgaactcttagagcaacaaaagcgtggatatattcagaagattttttctcaagatttaagatttaaagatgaaaatggaaacagttatcctgattggtctattaaaaagattgaag

SEQ ID NO: 11 - DNA, 1200 bp, Staphylococcus aureus
accattttagctgtagggaaactaaaagagaaatattggaagcaagccatagcagaatatgaaaaacgtttaggcccatacaccaagatagacatcatagaagttccagacgaaaaagcaccagaaaatatgagcgacaaagaaattgagcaagtaaaagaaaaagaaggccaacgaatactagccaaaattaaaccacaatccacagtcattacattagaaatacaaggaaagatgctatcttccgaaggattggcccaagaattgaaccaacgcatgacccaagggcaaagcgactttgtattcgtcattggcggatcaaacggcctgcacaaggacgtcttacaacgcagtaactacgcactatcattcagcaaaatgacattcccacatcaaatgatgcgggttgtgttaattgagcaagtgtatagagcatttaagattatgcgtggagaagcatatcataaatgatgcggttttttcagccgcttcataaagggattttgaatgtatcagaacatatgaggtttatgtgaattgctgttatgtttttaagaagcatatcataaatgatgcggttttttcagccgcttcataaagggattttgaatgtatcagaacatatgaggtttatgtgaattgctgttatgtttttaagaagcatatcataagtgatgcggtttttattaattagttgctaaaaaatgaagtatgcaatattaattattattaaattttgatatatttaaagaaagattaagtttagggtgaatgaatggcttatcaaagtgaatatgcattagaaaatgaagtacttcaacaacttgaggaattgaactatgaaagagtaaatatacataatattaaattagaaattaatgaatatctcaaagaactaggagtgttgaaaaatgaataagcagacaaatactccagaactaagatttccagagtttgatgaggaatggaaaaaaaggaaattaggtgaagtagtaaattataaaaatggtggttcatttgaaagtttagtgaaaaaccatggtgtatataaactcataactcttaaatctgttaatacagaaggaaagttgtgtaattctggaaaatatatcgatgataaatgtgttgaaacattgtgtaatgatactttagtaatgatactgagcgagcaagcaccaggactagttggaatgactgcaa

SEQ ID NO: 12 - DNA, 1017 bp, Staphylococcus aureus
aacgtttaggcccatacaccaagatagacatcatagaagttccagacgaaaaagcaccagaaaatatgagcgacaaagaaatcgagcaagtaaaagaaaaagaaggccaacgaatactagccaaaatcaaaccacaatccacagtcattacattagaaatacaaggaaagatgctatcttccgaaggattggcccaagaattgaaccaacgcatgacccaagggcaaagcgactttgtattcgtcattggcggatcaaacggcctgcacaaggacgtcttacaacgcagtaactacgcactatcattcagcaaaatgacattcccacatcaaatgatgcgggttgtgttaattgaagcaagtgtatagagcgtttaagattatgcgcggagaagcgtatcacaaatgatgcggtttttttaacctctttacgtatgaggtttatgagaattgccgttatgttttgcgagagttatcaatctttttgatagtaagaaagtacatagaaactaaaagagtatttttatctacaatagcatttataatttattctattattgtatacttattttaattattagtatcattgctgagatgttacttgatattctatgtctattttttaggaaattctatactattaaaattatggtattttatacgcaataaaggactaatctattttatacagattagtcctttattgtagtctttaaaaactagttactcattaatattttttagtacaatttcagcaacctcacttactattttgtcattaggtttaccatcttttctatctttatttgtaaatatcaccagaattataggtttatcttgtccatctggataaacaaagcgaacatcgtttcttgaaccgtatgttagtgcttgaccgctcttatccataactttaaagtttgaaggtgcaccatccttaattaatgtatcgccacttttatttttgaacattagattaagtaagaaatctttgtttgctttgctaagatctccatca

SEQ ID NO: 13 - DNA, 2207 bp, Staphylococcus aureus
ccttctacacctccatatcacaaaaattataacattattttgacataaatactacatttgtaatatactacaaatgtagtcttatataaggaggatattgatgaaaaagataaaaattgttccacttattttaatagttgtagttgtcgggtttggtatatatttttatgcttccaaagataaagaaattaataatactattgatgcaattgaagataaaaatttcaaacaagtttataaagatagcagttatatttctaaaagcgataatggtgaagtagaaatgactgaacgtccgataaaaatatataatagtttaggcgttaaagatataaacattcaggatcgtaaaataaaaaaagtatctaaaaataaaaaacgagtagatgctcaatataaaattaaaacaaactacggtaacattgatcgcaacgttcaatttaattttgttaaagaagatggtatgtggaagttagattgggatcatagcgtcattattccaggaatgcagaaagaccaaagcatacatattgaaaatttaaaatcagaacgtggtaaaattttagaccgaaacaatgtggaattggccaatacaggaacagcatatgagataggcatcgttccaaagaatgtatctaaaaaagattataaagcaatcgctaaagaactaagtatttctgaagactatatcaaacaacaaatggatcaaaattgggtacaagatgataccttcgttccacttaaaaccgttaaaaaaatggatgaatatttaagtgatttcgcaaaaaaatttcatcttacaactaatgaaacagaaagtcgtaactatcctctaggaaaagcgacttcacatctattaggttatgttggtcccattaactctgaagaattaaaacaaaaagaatataaaggctataaagatgatgcagttattggtaaaaagggactcgaaaaactttacgataaaaagctccaacatgaagatggctatcgtgtcacaatcgttgacgataatagcaatacaatcgcacatacattaatagagaaaaagaaaaaagatggcaaagatattcaactaactattgatgctaaagttcaaaagagtatttataacaacatgaaaaatgattatggctcaggtactgctatccaccctcaaacaggtgaattattagcacttgtaagcacaccttcatatgacgtctatccatttatgtatggcatgagtaacgaagaatataataaattaaccgaagataaaaaagaacctctgctcaacaagttccagattacaacttcaccaggttcaactcaaaaaatattaacagcaatgattgggttaaataacaaaacattagacgataaaacaagttataaaatcgatggtaaaggttggcaaaaagataaatcttggggtggttacaacgttacaagatatgaagtggtaaatggtaatatcgacttaaaacaagcaatagaatcatcagataacattttctttgctagagtagcactcgaattaggcagtaagaaatttgaaaaaggcatgaaaaaactaggtgttggtgaagatataccaagtgattatccattttataatgctcaaatttcaaacaaaaatttagataatgaaatattattagctgattcaggttacggacaaggtgaaatactgattaacccagtacagatcctttcaatctatagcgcattagaaaataatggcaatattaacgcacctcacttattaaaagacacgaaaaacaaagtttggaagaaaaatattatttccaaagaaaatatcaatctattaactgatggtatgcaacaagtcgtaaataaaacacataaagaagatatttatagatcttatgcaaacttaattggcaaatccggtactgcagaactcaaaatgaaacaaggagaaactggcagacaaattgggtggtttatatcatatgataaagataatccaaacatgatgatggctattaatgttaaagatgtacaagataaaggaatggctagctacaatgccaaaatctcaggtaaagtgtatgatgagctatatgagaacggtaataaaaaatacgatatagatgaataacaaaacagtgaagcaatccgtaacgatggttgcttcactgttttattatgaattattaataagtgctgttacttctcccttaaatacaatttcttcattt

SEQ ID NO: 14 - DNA, 1998 bp, Staphylococcus aureus
atgaaaaaaatttatattagtgtgctagttcttttactaattatgattataataacttggttattcaaagatgacgatattgagaaaacaattagttctattgaaaaaggaaactataacgaagtatataaaaatagttcagaaaaatctaaactggcatatggagaagaagaaattgtagataggaataaaaaaatttacaaagatttaagtgtcaataacttaaaaattactaatcatgaaattaaaaaaactggaaaagataaaaagcaagttgatgttaaatataacatatatacaaaatatggaactatacgacgtaatacacaattaaactttatttatgaagataagcattggaaattagattggagaccagacgtaatagtacctggtttgaaaaatggacagaaaattaatatagaaacattaaaatcagagcgaggcaaaataaaagatagaaatggtatagaattagctaaaactggaaatacatatgaaatcggtattgtccctaacaaaacacccaaagaaaaatatgatgatattgctcgtgacttacaaattgatacaaaagctataaccaataaagttaatcaaaaatgggttcagccagattcatttgtaccaattaaaaagataaataaacaagatgaatatatagacaaattaattaaatcatacaatttacaaataaacactataaaaagccgtgtttatccattgaacgaagcaacagtacaccttttaggttatgtgggtccaattaattctgacgagttaaaaagtaagcaatttagaaactatagcaaaaatactgttattggaaaaaaaggcttagaacgcctctatgataaacaattgcaaaacactgatggttttaaggtatccattgcaaatacttatgacaataaacctttagacacattattggagaaaaaggctgaaaacggaaaagatcttcatttaactatagatgctagagtacaagaaagtatttataaacatatgaaaaatgacgatggatctggtacagcattacaaccaaaaactggagaaattttagctttggtaagtaccccatcgtacgatgtttatccattcatgaatggattaagcaataatgactaccgtaaattaactaacaataaaaaagagcctttgctcaacaaatttcaaatcactacatcaccaggttcaacccaaaaaatattaacatctattatagccttaaaagaaaataaactagacaaaaatactaattttgatatttatggtaagggttggcaaaaagatgcatcatgggggaattataatatcacaagatttaaagtagtagacggcaatatcgatttaaagcaagcaatagaatcatcagacaacatattttttgcccgcattgcattagcattaggagccaaaaaatttgagcaaggtatgcaagatttgggaatcggtgaaaatatcccgagtgattatcccttttataaagcacaaatctcaaatagtaatttaaaaaatgaaatattattagcagattcaggatatggccaaggcgagatactagtaaaccctatacaaattttatcaatatacagtgctttagaaaataacggaaatatacaaaatcctcatgttttacgtaaaacaaaatctcaaatatggaaaaaagatattatacctaaaaaagacatagatatattaactaatggtatggaacgtgtagttaataaaacacatagggatgatatatacaaaaattatgcccgaattattggtaaatctggcacagcagaattaaaaatgaatcaaggggaaactggaagacaaataggttggtttgtttcatataataaaaataatcctaatatgttaatggcgattaatgttaaagacgttcaaaataaagggatggccagctataatgctactatatctggaaaagtttatgatgatttgtatgataatggaaaaactcaatttgatatagatcagtaa

SEQ ID NO: 15 - DNA, 1011 bp, Staphylococcus aureus
atggcagtaaaagtagcaattaatggttttggtagaattggtcgtttagcattcagaagaattcaagaagtagaaggtcttgaagttgtagcagtaaacgacttaacagatgacgacatgttagcgcatttattaaaatatgacactatgcaaggtcgtttcacaggtgaagtagaggtagttgatggtggtttccgcgtaaatggtaaagaagttaaatcattcagtgaaccagatgcaagcaaattaccttggaaagacttaaatatcgatgtagtattagaatgtactggtttctacactgataaagataaagcacaagctcatattgaagcaggcgctaaaaaagtattaatctcagcaccagctactggtgacttaaaaacaatcgtattcaacactaaccaccaagagttagacggttctgaaacagttgtttcaggtgcttcatgtactacaaactcattagcaccagttgctaaagttttaaacgatgactttggtttagttgaaggtttaatgactacaattcacgcttacacaggtgatcaaaatacacaagacgcacctcacagaaaaggtgacaaacgtcgtgctcgtgcagcggcagaaaacatcatccctaactcaacaggtgctgctaaagctatcggtaaagttattcctgaaatcgatggtaaattagatggtggtgcacaacgtgttcctgtagctacaggttcattaactgaattaacagtagtattagaaaaacaagacgtaacagttgaacaagttaacgaagctatgaaaaatgcttcaaacgaatcattcggttacactgaagacgaaatcgtttcttcagacgttgtaggtatgacttacggttcattattcgacgctacacaaactcgtgtaatgtcagttggcgaccgtcaattagttaaagttgcagcttggtatgataacgaaatgtcatatactgcacaattagttcgtacattagcatacttagctgaactttctaaataa

SEQ ID NO: 16 - DNA, 356 bp, Staphylococcus aureus
aacgtttaggcccatacaccaagatagacatcatagaagttccagacgaaaaagcaccagaaaatatgagcgacaaagaaatcgagcaagtaaaagaaaaagaaggccaacgaatactagccaaaatcaaaccacaatccacagtcattacattagaaatacaaggaaagatgctatcttccgaaggattggcccaagaattgaaccaacgcatgacccaagggcaaagcgactttgtattcgtcattggcggatcaaacggcctgcacaaggacgtcttacaacgcagtaactacgcactatcattcagcaaaatgacattcccacatcaaatgatgcgggttgtgttaattgaa

SEQ ID NO: 17 - DNA, 819 bp, Staphylococcus aureus
aacgtttaggcccatacaccaagatagacatcatagaagttccagacgaaaaagcaccagaaaatatgagcgacaaagaaatcgagcaagtaaaagaaaaagaaggccaacgaatactagccaaaatcaaaccacaatccacagtcattacattagaaatacaaggaaagatgctatcttccgaaggattggcccaagaattgaaccaacgcatgacccaagggcaaagcgactttgtattcgtcattggcggatcaaacggcctgcacaaggacgtcttacaacgcagtaactacgcactatcattcagcaaaatgacattcccacatcaaatgatgcgggttgtgttaattgaacaagtgtatagagcatttaagattatgcgaggagaagcgtatcacaaataaaactaaaaaatagattgtgtataatataaaaggaagggatttatattaaaattttgaattcaaaaattattgaaagggaagctaccttagaaattgaatctatggccactaatacattgaaaataaacccagacattaattcttactatacagaaatgtctttcgatggagaattggaagtgtatgatcctgaaaatttgaataaaaaatttcgttggaaaaatacaagttcaagttaaaggaaaagaagtagctaaaagaggaggtaagattattcgtcgaagtaatgggttctgttgcaaagtaaaaaaatatagctaaccactaatttatcatgtcagtgttcgcttaacgatataaatagctccattttccttttattttgatgtacgtctcatcaatacgccatttg

SEQ ID NO: 18 - DNA, 868 bp, Staphylococcus aureus
accattttagctgtagggaaactaaaagagaaatattggaagcaagccatagcagaatatgaaaaacgtttaggcccatacaccaagatagacatcatagaagttccagacgaaaaagcaccagaaaatatgagtgacaaagaaattgagcaagtaaaagaaaaagaaggccaacgaatactagccaaaatcaaaccacaatccacagtcattacattagaaatacaaggaaagatgctatcttccgaaggattggcccaagaattgaaccaacgcatgacccaagggcaaagcgactttgttttcgtcattggcggatcaaacggcctgcacaaggacgtcttacaacgcagtaactacgcactatcattcagcaaaatgacattcccacatcaaatgatgcgggttgtgttaattgaacaagtgtacagagcatttaagattatgcgaggagaagcgtatcacaaataaaactaaaaaatagattgtgtataatataaaaggagcggatttatattaaaactttgaattcaaaaattattgaaagggaagctaccttagaaattgaatctatggcaactaatacattgaaaataaacccggatattaattcaaacgatacaaaaatgtctttcgatggagaattggaagtgtatgattctgaaaatttgagtaaaaaaaatttcgttggaaaaatacaagttcaagttaaaggaaaggaagtagctaaaagaggaggtaaggttattcatcgaagtaatgtcaaaatgaatgatttaaaggcataccaacgagaaggtggtgtgtattactttgtcgtgtatttaatcgttgagaataaaaaagttgttgagaagcaggtttatgg

SEQ ID NO: 19 - DNA, 36 bp, Artificial Sequence
  GAPDH FRET Cassette
  misc_feature (1)..(1): Cal Fluor Red 610 labeled
  misc_feature (4)..(4): Black Hole Quencher 2-dT
  misc_feature (35)..(35): 3'-terminal Hexanediol
tcttagccggttttccggctgagactccgcgtccgt

SEQ ID NO: 20 - DNA, 24 bp, Artificial Sequence
  GAPDH Forward amplification oligomer
cgtttcacaggtgaagtagaggta

SEQ ID NO: 21 - DNA, 29 bp, Artificial Sequence
  GAPDH Reverse amplification oligomer
  modified_base (1)..(29): n = 5'-methyl-2'deoxycytosine
  misc_feature (2)..(2): n is a, c, g, or t
  misc_feature (7)..(7): n is a, c, g, or t
  misc_feature (11)..(11): n is a, c, g, or t
  misc_feature (17)..(17): n is a, c, g, or t
  misc_feature (20)..(20): n is a, c, g, or t
  misc_feature (23)..(23): n is a, c, g, or t
cnagtanattntaatantanatngatatt

SEQ ID NO: 22 - DNA, 30 bp, Artificial Sequence
  GAPDH detection oligomer
  misc_feature (30)..(30): 3'-terminal Hexanediol
acggacgcggagagttgatggtggtttccg

SEQ ID NO: 23 - DNA, 32 bp, Artificial Sequence
  GAPDH Forward amplification oligomer
cgcgtaaatggtaaagaagttaaatcattcag

SEQ ID NO: 24 - DNA, 27 bp, Artificial Sequence
  GAPDH Reverse amplification oligomer
gagcttgtgctttatctttatcagtgt

SEQ ID NO: 25 - DNA, 30 bp, Artificial Sequence
  GAPDH detection oligomer
  misc_feature (30)..(30): 3'-terminal Hexanediol
acggacgcggaggtgaaccagatgcaagca

SEQ ID NO: 26 - DNA, 26 bp, Artificial Sequence
  GAPDH Reverse amplification oligomer
ctgtttcagaaccgtctaactcttgg

SEQ ID NO: 27 - DNA, 35 bp, Artificial Sequence
  mecA/C FRET Cassette
  misc_feature (1)..(1): Hexochloro-Fluorescein labeled
  misc_feature (4)..(4): Blackberry Quencher 650 dT
  misc_feature (35)..(35): 3'-terminal Hexanediol
tctagccggttttccggctgagacgtccgtggcct

SEQ ID NO: 28 - DNA, 43 bp, Artificial Sequence
  mecC detection oligomer
  misc_feature (43)..(43): 3'-terminal Hexanediol
acggacgcggagcatctattatagccttaaaagaaaataaact

SEQ ID NO: 29 - DNA, 38 bp, Artificial Sequence
  mecA detection oligomer
  misc_feature (38)..(38): 3'-terminal Hexanediol
acggacgcggagtcgattttataacttgttttatcgtc

SEQ ID NO: 30 - DNA, 25 bp, Artificial Sequence
  mecA/C Forward amplification oligomer
ttatctttttgccaacctttaccat

SEQ ID NO: 31 - DNA, 29 bp, Artificial Sequence
  mecA/C Reverse amplification oligomer
tcaccaggttcaactcaaaaaatattaac

SEQ ID NO: 32 - DNA, 43 bp, Artificial Sequence
  mecC detection oligomer
  misc-feature (43)..(43): 3'-terminal Hexanediol
aggccacggacgcatctattatagccttaaaagaaaataaact

SEQ ID NO: 33 - DNA, 38 bp, Artificial Sequence
  mecA detection oligomer
  misc_feature (38)..(38): 3'-terminal Hexanediol
aggccacggacgtcgattttataacttgttttatcgtc

SEQ ID NO: 34 - DNA, 23 bp, Artificial Sequence
  mecA/C Forward amplification oligomer
  mod_base (1)..(23): n = 5'-methyl-2'deoxycytosine
  misc_feature (3)..(3): n is a, c, g, or t
  misc_feature (10)..(11): n is a, c, g, or t
  misc_feature (14)..(15): n is a, c, g, or t
  misc_feature (20)..(21): n is a, c, g, or t
atntttttgnnaanntttannat

SEQ ID NO: 35 - DNA, 29 bp, Artificial Sequence
  mecA/C Reverse amplification oligomer
  mod_base (1)..(29): n = 5'-methyl-2'deoxycytosine
  misc_feature (2)..(2): n is a, c, g, or t
  misc_feature (4)..(5): n is a, c, g, or t
  misc_feature (11)..(11): n is a, c, g, or t
  misc_feature (14)..(14): n is a, c, g, or t
  misc_feature (16)..(16): n is a, c, g, or t
tnannaggttnaantnaaaaaatattaac

SEQ ID NO: 36 - DNA, 35 bp, Artificial Sequence
  mecA/C Forward amplification oligomer
gcaaagaaaatgttgtctgatgattctattgcttg

SEQ ID NO: 37 - DNA, 30 bp, Artificial Sequence
  mecA/C Forward amplification oligomer
gaaaatgttgtctgatgattctattgcttg

SEQ ID NO: 38 - DNA, 30 bp, Artificial Sequence
  mecA Reverse amplification oligomer
cttggggtggttacaacgttacaagatatg

SEQ ID NO: 39 - DNA, 26 bp, Artificial Sequence
  mecA/C Forward amplification oligomer
cctgaatctgctaataatatttcatt

SEQ ID NO: 40 - DNA, 22 bp, Artificial Sequence
  mecA forward amplification oligomer
gtgtcttttaataagtgaggtg

SEQ ID NO: 41 - DNA, 29 bp, Artificial Sequence
  mecA detection oligomer
  misc_feature (29)..(29): 3'-terminal Hexanediol
aggccacggacgcgtaacctgaatcagct

SEQ ID NO: 42 - DNA, 26 bp, Artificial Sequence
  mecA Invader
gggttaatcagtatttcaccttgtca

SEQ ID NO: 43 - DNA, 28 bp, Artificial Sequence
  mecA detection oligomer
  misc_feature (28)..(28): 3'-terminal Hexanediol
aggccacggacgcaccttgtccgtaacc

SEQ ID NO: 44 - DNA, 28 bp, Artificial Sequence
  mecA 449-465 (+) Invader
ggatctgtactgggttaatcagtattta

SEQ ID NO: 45 - DNA, 20 bp, Artificial Sequence
  mecA reverse amplification oligomer
ggtgttggtgaagatatacc

SEQ ID NO: 46 - DNA, 24 bp, Artificial Sequence
  mecC Invader
atcactcgggatattttcaccgac

SEQ ID NO: 47 - DNA, 30 bp, Artificial Sequence
  mecC detection oligomer
acggacgcggagttcccaaatcttgcatac

SEQ ID NO: 48 - DNA, 26 bp, Artificial Sequence
  mecC reverse amplification oligomer
ttaaagcaagcaatagaatcatcaga

SEQ ID NO: 49 - DNA, 21 bp, Artificial Sequence
  mecC reverse amplification oligomer
atggtaagggttggcaaaaag

SEQ ID NO: 50 - DNA, 20 bp, Artificial Sequence
  MREJ i Reverse amplification oligomer
gaaagactgcggaggctaac

SEQ ID NO: 51 - DNA, 22 bp, Artificial Sequence
  MREJ i Reverse amplification oligomer
gctaactatgtcaaaaatcatg

SEQ ID NO: 52 - DNA, 22 bp, Artificial Sequence
  MREJ i Reverse amplification oligomer
gactgcggaggctaactatgtc

SEQ ID NO: 53 - DNA, 19 bp, Artificial Sequence
  MREJ ii, viii, ix, xiv Reverse amplification oligomer
aagcggctgaaataaccgc

SEQ ID NO: 54 - DNA, 19 bp, Artificial Sequence
  MREJ ii, viii, ix, xiv Reverse amplification oligomer
aagcggctgaaaaaaccgc

SEQ ID NO: 55 - DNA, 18 bp, Artificial Sequence
  MREJ ii Reverse amplification oligomer
  mod_base (1)..(18): n = = 5'-methyl-2'deoxycytosine
  misc_feature (2)..(3): n is a, c, g, or t
  misc_feature (13)..(13): n is a, c, g, or t
  misc_feature (16)..(16): n is a, c, g, or t
cnntttatgaagnggntg

SEQ ID NO: 56 - DNA, 19 bp, Artificial Sequence
  MREJ v Reverse amplification oligomer
ttacggctgaaataaccgc

SEQ ID NO: 57 - DNA, 20 bp, Artificial Sequence
  MREJ xxi Reverse amplification oligomer
ctctcgcaaaacataacggc

SEQ ID NO: 58 - DNA, 33 bp, Artificial Sequence
  orfX/SCCmec junction FRET Cassette
  misc_feature (1)..(1): Fluorescein labeled
  misc_feature (4)..(4): Blackberry Quencher 650 dT labeled
  misc_feature (33)..(33): 3'-terminal Hexanediol
tctagccggttttccggctgagacctcggcgcg

SEQ ID NO: 59 - DNA, 16 bp, Artificial Sequence
  orfX Forward amplification oligomer
cttccgaaggattggc

SEQ ID NO: 60 - DNA, 23 bp, Artificial Sequence
  orfX Forward amplification oligomer
ccgaaggattggcccaagaattg

SEQ ID NO: 61 - DNA, 29 bp, Artificial Sequence
  orfX/SCCmec junction detection oligomer
  modified_base (12)..(12): I
  misc_feature (12)..(12): n is a, c, g, or t
  misc_feature (29)..(29): 3'-terminal Hexanediol
cgcgccgaggcncaagaattgaaccaacg

SEQ ID NO: 62 - DNA, 26 bp, Artificial Sequence
  orfX/SCCmec junction detection oligomer
  misc_feature (26)..(26): 3'-terminal Hexanediol
cgcgccgagggaaccaacgcatgacc

SEQ ID NO: 63 - DNA, 22 bp, Artificial Sequence
  MREJ iv Reverse amplification oligomer
ggatatggaaatccatctctac

SEQ ID NO: 64 - DNA, 34 bp, Artificial Sequence
  MREJ iv Reverse amplification oligomer
cgctactaaagaggatatggaaatccatctctac

SEQ ID NO: 65 - DNA, 22 bp, Artificial Sequence
  MREJ iv Reverse amplification oligomer
  mod_base (1)..(2): n = 5'-methyl-2'deoxycytosine
  misc_feature (2)..(3): n is a, c, g, or t
  misc_feature (5)..(5): n is a, c, g, or t
  misc_feature (8)..(8): n is a, c, g, or t
anngntantaaagaggatatgg

SEQ ID NO: 66 - DNA, 19 bp, Artificial Sequence
  MREJ v Reverse amplification oligomer
  mod_base (1)..(19): n = 5'-methyl-2'deoxycytosine
  misc_feature (4)..(4): n is a, c, g, or t
  misc_feature (7)..(7): n is a, c, g, or t
  misc_feature (17)..(17): n is a, c, g, or t
ttanggntgaaataacngc

SEQ ID NO: 67 - DNA, 28 bp, Artificial Sequence
  MREJ vi Reverse amplification oligomer
ctgattttcactcttcatctacttactc

SEQ ID NO: 68 - DNA, 26 bp, Artificial Sequence
  MREJ vi Reverse amplification oligomer
gatataggtgtcacatcatatttcgc

SEQ ID NO: 69 - DNA, 32 bp, Artificial Sequence
  MREJ xiii Reverse amplification oligomer
ctctttcatagttcaattcctcaagttgttga

SEQ ID NO: 70 - DNA, 25 bp, Artificial Sequence
  MREJ xiii Reverse amplification oligomer
  mod_base (1)..(25): n = 5'-methyl-2'deoxycytosine
  misc_feature (10)..(10): n is a, c, g, or t
  misc_feature (13)..(13): n is a, c, g, or t
  misc_feature (19)..(19): n is a, c, g, or t
gttgaagtanttnattttntaatgc

SEQ ID NO: 71 - DNA, 30 bp, Artificial Sequence
  MREJ xiii Reverse amplification oligomer
gccattcattcaccctaaacttaatctttc

SEQ ID NO: 72 - DNA, 19 bp, Artificial Sequence
  MREJ xiii Reverse amplification oligomer
ccattcattcaccctaaac

SEQ ID NO: 73 - DNA, 20 bp, Artificial Sequence
  MREJ iii Reverse amplification oligomer
atacacaacctaatttttag

SEQ ID NO: 74 - DNA, 24 bp, Artificial Sequence
  MREJ iii Reverse amplification oligomer
gtatgatattgcaaggtataatcc

SEQ ID NO: 75 - DNA, 30 bp, Artificial Sequence
  MREJ iii Reverse amplification oligomer
cactctataaacatcgtatgatattgcaag

SEQ ID NO: 76 - DNA, 30 bp, Artificial Sequence
  MREJ vii Reverse amplification oligomer
taatggaaattcttaatctttacttgtacc

SEQ ID NO: 77 - DNA, 26 bp, Artificial Sequence
  MREJ vii Reverse amplification oligomer
  mod_base (1)..(26): n = 5'-methyl-2'deoxycytosine
  misc_feature (8)..(8): n is a, c, g, or t
  misc_feature (14)..(14): n is a, c, g, or t
  misc_feature (19)..(19): n is a, c, g, or t
  misc_feature (25)..(25): n is a, c, g, or t
ggaaattnttaatntttanttgtanc

SEQ ID NO: 78 - DNA, 27 bp, Artificial Sequence
  MREJ vii Reverse amplification oligomer
caaaaagaagtcgatttacacaccatg

SEQ ID NO: 79 - DNA, 31 bp, Artificial Sequence
  MREJ vii Reverse amplification oligomer
ctttacatcgcttactgcaaacatctaatac

SEQ ID NO: 80 - DNA, 25 bp, Artificial Sequence
  MREJ xii Reverse amplification oligomer
  mod_base (1)..(25): n = 5'-methyl-2'deoxycytosine
  misc_feature (7)..(7): n is a, c, g, or t
  misc_feature (13)..(14): n is a, c, g, or t
  misc_feature (16)..(16): n is a, c, g, or t
  misc_feature (18)..(20): n is a, c, g, or t
aatgagntttttnnantnnnatttc

SEQ ID NO: 81 - DNA, 18 bp, Artificial Sequence
  MREJ xii Reverse amplification oligomer
  mod_base (1)..(18): n = 5'-methyl-2'deoxycytosine
  misc_feature (2)..(3): n is a, c, g, or t
  misc_feature (5)..(5): n is a, c, g, or t
  misc_feature (7)..(9): n is a, c, g, or t
  misc_feature (14)..(14): n is a, c, g, or t
  misc_feature (17)..(17): n is a, c, g, or t
tnnantnnnatttnttnc

SEQ ID NO: 82 - DNA, 22 bp, Artificial Sequence
  MREJ xii Reverse amplification oligomer
acttaatgagctttttccactc

SEQ ID NO: 83 - DNA, 25 bp, Artificial Sequence
  MREJ xv Reverse amplification oligomer
  mod_base (1)..(25): n = 5'-methyl-2'deoxycytosine
  misc_feature (7)..(7): n is a, c, g, or t
  misc_feature (16)..(16): n is a, c, g, or t
  misc_feature (19)..(21): n is a, c, g, or t
caatttntaaggtagnttnnntttc

SEQ ID NO: 84 - DNA, 25 bp, Artificial Sequence
  MREJ xv Reverse amplification oligomer
caatttctaaggtagcttccctttc

SEQ ID NO: 85 - DNA, 12 bp, Artificial Sequence
  orfX/SCCmec junctiondetection oligomer core sequence
ccgagggaacca

SEQ ID NO: 86 - DNA, 12 bp, Artificial Sequence
  orfX/SCCmec junctiondetection oligomer core sequence
  mod_base (8)..(8): I
  misc_feature (8)..(8): n is a, c, g, or t
ccgaggcncaag

SEQ ID NO: 87 - DNA, 12 bp, Artificial Sequence
  mecA detection oligomer core sequence
cggacgtcgatt

SEQ ID NO: 88 - DNA, 12 bp, Artificial Sequence
  mecA detection oligomer core sequence
caacctgtttta

SEQ ID NO: 89 - DNA, 12 bp, Artificial Sequence
  mecA detection oligomer core sequence
gcggagtcgatt

SEQ ID NO: 90 - DNA, 12 bp, Artificial Sequence
  mecA detection oligomer core sequence
cggacgcgtaac

SEQ ID NO: 91 - DNA, 12 bp, Artificial Sequence
  mecA detection oligomer core sequence
cggacgcacctt

SEQ ID NO: 92 - DNA, 12 bp, Artificial Sequence
  mecC detection oligomer core sequence
gcggagcatcta

SEQ ID NO: 93 - DNA, 12 bp, Artificial Sequence
  mecC detection oligomer core sequence
gcggagttccca

SEQ ID NO: 94 - DNA, 12 bp, Artificial Sequence
  mecC detection oligomer core sequence
cggacgcatcta

SEQ ID NO: 95 - DNA, 12 bp, Artificial Sequence
  GAPDH detection oligomer core sequence
gcggaggtgaac

SEQ ID NO: 96 - DNA, 12 bp, Artificial Sequence
  GAPDH detection oligomer core sequence
gcggagagttga

SEQ ID NO: 97 - DNA, 16 bp, Artificial Sequence
  orfX/SCCmec junctiondetection oligomer target-hybridizing sequence
gaaccaacgcatgacc

SEQ ID NO: 98 - DNA, 19 bp, Artificial Sequence
  orfX/SCCmec junctiondetection oligomer target-hybridizing sequence
  mod_base (2)..(2): I
  misc_feature (2)..(2): n is a, c, g, or t
cncaagaattgaaccaacg

SEQ ID NO: 99 - DNA, 26 bp, Artificial Sequence
  mecA detection oligomer target-hybridizing sequence
tcgattttataacttgttttatcgtc

SEQ ID NO: 100 - DNA, 26 bp, Artificial Sequence
  mecA detection oligomer target-hybridizing sequence
tcgattttataacttgttttatcgtc

SEQ ID NO: 101 - DNA, 28 bp, Artificial Sequence
  mecA detection oligomer target-hybridizing sequence
gttttaagtcgatattaccatttaccac

SEQ ID NO: 102 - DNA, 17 bp, Artificial Sequence
  mecA detection oligomer target-hybridizing sequence
cgtaacctgaatcagct

SEQ ID NO: 103 - DNA, 16 bp, Artificial Sequence
  mecA detection oligomer target-hybridizing sequence
caccttgtccgtaacc

SEQ ID NO: 104 - DNA, 31 bp, Artificial Sequence
  mecC detection oligomer target-hybridizing sequence
catctattatagccttaaaagaaaataaact

SEQ ID NO: 105 - DNA, 31 bp, Artificial Sequence; identical to SEQ ID NO: 104
  mecC detection oligomer target-hybridizing sequence

SEQ ID NO: 106 - DNA, 18 bp, Artificial Sequence
  mecC detection oligomer target-hybridizing sequence
ttcccaaatcttgcatac

SEQ ID NO: 107 - DNA, 18 bp, Artificial Sequence
  GAPDH detection oligomer target-hybridizing sequence
gtgaaccagatgcaagca

SEQ ID NO: 108 - DNA, 18 bp, Artificial Sequence
  GAPDH detection oligomer target-hybridizing sequence
agttgatggtggtttccg

SEQ ID NO: 109 - DNA, 23 bp, Artificial Sequence
  mecC forward amplification oligomer
atctttttgccaacccttaccat

SEQ ID NO: 110 - DNA, 29 bp, Artificial Sequence
  mecC reverse amplification oligomer
tcaccaggttcaacccaaaaaatattaac

SEQ ID NO: 111 - DNA, 28 bp, Artificial Sequence
  orfX/SCCmec junctiondetection oligomer
acggacgcggaggaaccaacgcatgacc

SEQ ID NO: 112 - DNA, 36 bp, Artificial Sequence
  mecA detection oligomer
cgcgccgaggtcgattttataacttgttttatcgtc

SEQ ID NO: 113 - DNA, 41 bp, Artificial Sequence
  mecC detection oligomer
cgcgccgaggcatctattatagccttaaaagaaaataaact

SEQ ID NO: 114 - DNA, 30 bp, Artificial Sequence
  GAPDH detection oligomer
aggccacggacggtgaaccagatgcaagca

SEQ ID NO: 115 - DNA, 28 bp, Artificial Sequence
  orfX/SCCmec junctiondetection oligomer
aggccacggacggaaccaacgcatgacc

SEQ ID NO: 116 - DNA, 38 bp, Artificial Sequence; identical to SEQ ID NO: 29
  mecA detection oligomer

SEQ ID NO: 117 - DNA, 43 bp, Artificial Sequence; identical to SEQ ID NO: 28
  mecC detection oligomer

SEQ ID NO: 118 - DNA, 28 bp, Artificial Sequence
  GAPDH detection oligomer
cgcgccgagggtgaaccagatgcaagca

SEQ ID NO: 119 - DNA, 12 bp, Artificial Sequence
  orfX/SCCmec junctiondetection oligomer core sequence
gcggaggaacca

SEQ ID NO: 120 - DNA, 12 bp, Artificial Sequence
  mecA detection oligomer core sequence
ccgaggtcgatt

SEQ ID NO: 121 - DNA, 12 bp, Artificial Sequence
  mecC detection oligomer core sequence
ccgaggcatcta

SEQ ID NO: 122 - DNA, 12 bp, Artificial Sequence
  GAPDH detection oligomer core sequence
cggacggtgaac

SEQ ID NO: 123 - DNA, 12 bp, Artificial Sequence
  orfX/SCCmec junctiondetection oligomer core sequence
cggacggaacca

SEQ ID NO: 124 - DNA, 12 bp, Artificial Sequence
  mecA detection oligomer core sequence
gcggagtcgatt

SEQ ID NO: 125 - DNA, 12 bp, Artificial Sequence
  mecC detection oligomer core sequence
gcggagcatcta

SEQ ID NO: 126 - DNA, 12 bp, Artificial Sequence
  GAPDH detection oligomer core sequence
ccgagggtgaac